European Patent Specification EP 3 831 404 B1, published January 28, 2026. Title: Antibodies that potently neutralize rabies virus and other lyssaviruses and uses thereof. Applicant: Humabs BioMed SA. The sequence listing filed with the application follows.

SEQUENCE LISTING (218 sequences)

SEQ ID NO: 1 - protein, 8 aa, Artificial Sequence
  RVA122 CDRH1 aa
GDSMNNFY

SEQ ID NO: 2 - protein, 7 aa, Artificial Sequence
  RVA122 CDRH2 aa
IYYSGTT

SEQ ID NO: 3 - protein, 17 aa, Artificial Sequence
  RVA122 CDRH3 aa
ARDSGDYVSYYYYGMDV

SEQ ID NO: 4 - protein, 8 aa, Artificial Sequence
  RVA122 CDRL1 aa
SSNIGSNY

SEQ ID NO: 5 - skipped

SEQ ID NO: 6 - protein, 9 aa, Artificial Sequence
  RVA122 CDRL2 long aa
LIYKSDKRP

SEQ ID NO: 7 - protein, 11 aa, Artificial Sequence
  RVA122 CDRL3 aa
AAWDNRLSGWL

SEQ ID NO: 8 - DNA, 24 bp, Artificial Sequence
  RVA122 CDRH1 nuc
ggtgactccatgaataatttctac

SEQ ID NO: 9 - DNA, 21 bp, Artificial Sequence
  RVA122 CDRH2 nuc
atctattacagtgggaccacc

SEQ ID NO: 10 - DNA, 51 bp, Artificial Sequence
  RVA122 CDRH3 nuc
gcgagagactccggtgactacgtcagctactactattatggtatggacgtc

SEQ ID NO: 11 - DNA, 24 bp, Artificial Sequence
  RVA122 CDRL1 nuc
agctccaacatcggaagtaattat

SEQ ID NO: 12 - skipped

SEQ ID NO: 13 - DNA, 27 bp, Artificial Sequence
  RVA122 CDRL2 long nuc
cttatttacaagagtgataagcggccc

SEQ ID NO: 14 - DNA, 33 bp, Artificial Sequence
  RVA122 CDRL3 nuc
gcagcatgggataacaggctgagtggttggctc

SEQ ID NO: 15 - protein, 123 aa, Artificial Sequence
  RVA122 heavy chain aa
QVHLQESGPGLVKPSETLSLTCTVSGDSMNNFYWGWIRQPAGKGLEWIGYIYYSGTTNYNPSLKSRVTISIDTSKNQFSLKVNSVTAADTAVYYCARDSGDYVSYYYYGMDVWGPGTTVTVSS

SEQ ID NO: 16 - protein, 110 aa, Artificial Sequence
  RVA122 light chain aa
QSVLTQSPSASDTPGQRVTISCSGSSSNIGSNYVYWYQQFPGTAPKLLIYKSDKRPSGVPDRFSGSTSGTSASLAISGLRSEDEADYYCAAWDNRLSGWLFGGGTKLTVL

SEQ ID NO: 17 - DNA, 370 bp, Artificial Sequence
  RVA122 heavy chain nuc
caggtgcacctgcaggagtcgggcccaggactggtgaagccttcggagaccctgtccctcacctgcactgtctctggtgactccatgaataatttctactggggctggatccggcagcccgcagggaagggactggagtggattggatatatctattacagtgggaccaccaactacaacccctccctcaagagtcgagtcaccatatcaatagacacgtccaagaaccaattctccctgaaggtgaactctgtgaccgctgcggacacggccgtgtattattgtgcgagagactccggtgactacgtcagctactactattatggtatggacgtctggggcccagggaccacggtcaccgtctcctcag

SEQ ID NO: 18 - DNA, 331 bp, Artificial Sequence
  RVA122 light chain nuc
cagtctgtgctgactcagtcaccctcagcgtctgatacccccgggcagagggtcaccatctcttgttctggaagcagctccaacatcggaagtaattatgtgtattggtaccagcagttcccaggaacggcccccaaactccttatttacaagagtgataagcggccctcaggggtccctgaccgattctctggctccacgtctggcacctcagcctccctggccatcagtgggctccggtccgaagatgaggctgattattactgtgcagcatgggataacaggctgagtggttggctcttcggcggagggacgaagctgaccgtcctag

SEQ ID NO: 19 - protein, 10 aa, Artificial Sequence
  RVA144 CDRH1 aa
GGSISSTIFY

SEQ ID NO: 20 - protein, 7 aa, Artificial Sequence
  RVA144 CDRH2 aa
VYYNGHT

SEQ ID NO: 21 - protein, 12 aa, Artificial Sequence
  RVA144 CDRH3 aa
ARPSTYDYSIGR

SEQ ID NO: 22 - protein, 9 aa, Artificial Sequence
  RVA144 CDRL1 aa
SSNIGAGYD

SEQ ID NO: 23 - skipped

SEQ ID NO: 24 - protein, 9 aa, Artificial Sequence
  RVA144 CDRL2 long aa
LIYGNTKRP

SEQ ID NO: 25 - protein, 11 aa, Artificial Sequence
  RVA144 CDRL3 aa
QSFDSSLSAWV

SEQ ID NO: 26 - DNA, 30 bp, Artificial Sequence
  RVA144 CDRH1 nuc
ggtggttccatcagcagtactattttctac

SEQ ID NO: 27 - DNA, 21 bp, Artificial Sequence
  RVA144 CDRH2 nuc
gtctattataatggacacacc

SEQ ID NO: 28 - DNA, 36 bp, Artificial Sequence
  RVA144 CDRH3 nuc
gcgagaccctcaacatatgactacagtattgggcgc

SEQ ID NO: 29 - DNA, 27 bp, Artificial Sequence
  RVA144 CDRL1 nuc
agctccaacatcggggcaggttatgat

SEQ ID NO: 30 - skipped

SEQ ID NO: 31 - DNA, 27 bp, Artificial Sequence
  RVA144 CDRL2 long nuc
ctcatctatggtaacaccaagcggccc

SEQ ID NO: 32 - DNA, 33 bp, Artificial Sequence
  RVA144 CDRL3 nuc
cagtcctttgacagcagcctgagtgcttgggta

SEQ ID NO: 33 - protein, 120 aa, Artificial Sequence
  RVA144 heavy chain aa
QLQLQESGPGLVKPSETLSLTCTVSGGSISSTIFYWGWIRQPPGKGLEWIGSVYYNGHTYYNPSLKSRVAISIDKSKNQFSLRLNSVTAADTAVYYCARPSTYDYSIGRWGQGTLVTVSS

SEQ ID NO: 34 - protein, 111 aa, Artificial Sequence
  RVA144 light chain aa
QSVLTQPPSVSRAPGQRVTISCTGSSSNIGAGYDVHWYQQLPGTAPKLLIYGNTKRPSGVPDRFSGSKSGTSASLAITGLLTEDEADYYCQSFDSSLSAWVFGGGTKLTVL

SEQ ID NO: 35 - DNA, 361 bp, Artificial Sequence
  RVA144 heavy chain nuc
cagctgcagctgcaggagtcgggcccaggactggtgaagccctcggagaccctgtccctcacttgcactgtctctggtggttccatcagcagtactattttctactggggctggatccgccagcccccagggaagggactggagtggattgggagtgtctattataatggacacacctactacaatccgtccctcaagagtcgagtcgccatatccattgacaagtccaagaaccagttctccctgaggcttaactctgtgaccgccgcggacacggctgtatattactgtgcgagaccctcaacatatgactacagtattgggcgctggggccagggaaccctggtcaccgtctcctcag

SEQ ID NO: 36 - DNA, 334 bp, Artificial Sequence
  RVA144 light chain nuc
cagtccgtgctgacgcagccgccctcagtgtctcgggccccagggcagagggtcaccatctcctgcactgggagcagctccaacatcggggcaggttatgatgtccactggtaccagcaacttccaggaacagcccccaaactcctcatctatggtaacaccaagcggccctcaggggtccctgaccgattctctggctccaagtctggcacctcagcctccctggccatcactgggctcctgactgaggatgaggctgattattactgccagtcctttgacagcagcctgagtgcttgggtattcggcggagggaccaaactgaccgtcctgg

SEQ ID NO: 37 - protein, 10 aa, Artificial Sequence
  RVB185 CDRH1 aa
GAPVSGVNSY

SEQ ID NO: 38 - protein, 7 aa, Artificial Sequence
  RVB185 CDRH2 aa
IKYSGST

SEQ ID NO: 39 - protein, 11 aa, Artificial Sequence
  RVB185 CDRH3 aa
ARQSTMTGRDY

SEQ ID NO: 40 - protein, 8 aa, Artificial Sequence
  RVB185 CDRL1 aa
RSNIGSHP

SEQ ID NO: 41 - skipped

SEQ ID NO: 42 - protein, 9 aa, Artificial Sequence
  RVB185 CDRL2 long aa
LIYGDSQRP

SEQ ID NO: 43 - protein, 12 aa, Artificial Sequence
  RVB185 CDRL3 aa
AAWDDSLSGLWV

SEQ ID NO: 44 - DNA, 30 bp, Artificial Sequence
  RVB185 CDRH1 nuc
ggtgcccccgtcagtggtgttaactcctac

SEQ ID NO: 45 - DNA, 21 bp, Artificial Sequence
  RVB185 CDRH2 nuc
atcaagtacagtgggagcacc

SEQ ID NO: 46 - DNA, 33 bp, Artificial Sequence
  RVB185 CDRH3 nuc
gccagacaaagtactatgacgggccgggactac

SEQ ID NO: 47 - DNA, 24 bp, Artificial Sequence
  RVB185 CDRL1 nuc
agatccaacatcggaagccatcct

SEQ ID NO: 48 - skipped

SEQ ID NO: 49 - DNA, 27 bp, Artificial Sequence
  RVB185 CDRL2 long nuc
ctcatctatggtgatagtcagcgaccc

SEQ ID NO: 50 - DNA, 36 bp, Artificial Sequence
  RVB185 CDRL3 nuc
gcagcatgggatgacagcctgagtggcctttgggtg

SEQ ID NO: 51 - protein, 119 aa, Artificial Sequence
  RVB185 heavy chain aa
QVQLQESGPGLVKPSETLSLTCSVSGAPVSGVNSYWVWIRQPPGKGLEWIATIKYSGSTHRSPSLRSRVTISVDTSKNQFSLELSSVTAADTAVYYCARQSTMTGRDYWGQGTLVTVSS

SEQ ID NO: 52 - protein, 111 aa, Artificial Sequence
  RVB185 light chain aa
QSVLTQPPSASGTPGQRVTISCSGSRSNIGSHPVNWYQQLPGAAPKLLIYGDSQRPSGVPDRFSGSKSGPSASLAISGLQSEDEADYYCAAWDDSLSGLWVFGGGTKLTVL

SEQ ID NO: 53 - DNA, 358 bp, Artificial Sequence
  RVB185 heavy chain nuc
caggtgcagctgcaggagtcgggcccaggactggtgaagccttcggagaccctgtccctcacctgcagtgtctccggtgcccccgtcagtggtgttaactcctactgggtgtggatccgccagccccccgggaaggggctggagtggattgcgactatcaagtacagtgggagcacccaccgtagcccgtcgctcaggagtcgagtcaccatatccgtagacacgtccaagaatcagttctccctggagctgagctctgtgaccgccgctgacacggctgtatattactgtgccagacaaagtactatgacgggccgggactactggggccagggaaccctggtcaccgtctcctcag

SEQ ID NO: 54 - DNA, 334 bp, Artificial Sequence
  RVB185 light chain nuc
cagtctgtgctgactcagccaccctcagcgtctgggacccccgggcagagggtcaccatctcttgttctggaagcagatccaacatcggaagccatcctgtaaactggtaccagcagctcccgggagcggcccccaagctcctcatctatggtgatagtcagcgaccctcaggggtccctgaccgattctctggctccaagtctggcccctcagcctccctggccatcagtggactccagtctgaagatgaggctgattattactgtgcagcatgggatgacagcctgagtggcctttgggtgttcggcggagggaccaagctgaccgtcctaa

SEQ ID NO: 55 - protein, 8 aa, Artificial Sequence
  RVB492 CDRH1 aa
GFSFSSYA

SEQ ID NO: 56 - protein, 8 aa, Artificial Sequence
  RVB492 CDRH2 aa
LNSIDHRT

SEQ ID NO: 57 - protein, 18 aa, Artificial Sequence
  RVB492 CDRH3 aa
ARGVGLWFGELSWNYFDY

SEQ ID NO: 58 - protein, 9 aa, Artificial Sequence
  RVB492 CDRL1 aa
SNDIGGYNY

SEQ ID NO: 59 - skipped

SEQ ID NO: 60 - protein, 9 aa, Artificial Sequence
  RVB492 CDRL2 long aa
MIFYVNKRP

SEQ ID NO: 61 - protein, 9 aa, Artificial Sequence
  RVB492 CDRL3 aa
CSFAGSYSL

SEQ ID NO: 62 - DNA, 24 bp, Artificial Sequence
  RVB492 CDRH1 nuc
ggattcagctttagcagctatgcc

SEQ ID NO: 63 - DNA, 24 bp, Artificial Sequence
  RVB492 CDRH2 nuc
cttaattctattgatcatagaaca

SEQ ID NO: 64 - DNA, 54 bp, Artificial Sequence
  RVB492 CDRH3 nuc
gctcggggggtgggactatggttcggtgaattatcctggaattactttgactac

SEQ ID NO: 65 - DNA, 27 bp, Artificial Sequence
  RVB492 CDRL1 nuc
agcaatgatattggtggttataactat

SEQ ID NO: 66 - skipped

SEQ ID NO: 67 - DNA, 27 bp, Artificial Sequence
  RVB492 CDRL2 long nuc
atgattttttatgtcaataagcggccc

SEQ ID NO: 68 - DNA, 27 bp, Artificial Sequence
  RVB492 CDRL3 nuc
tgctcatttgcaggcagttactcctta

SEQ ID NO: 69 - protein, 125 aa, Artificial Sequence
  RVB492 heavy chain variant 1 aa
EVQLMESGGGLVQPGGSMRLYCAASGFSFSSYAMSWVRQAPGKGLEWVSSLNSIDHRTDYADSVKGRFTISRDNSKNTLYLQMDSLRVEDSAMYYCARGVGLWFGELSWNYFDYWGQGTLVTVSS

SEQ ID NO: 70 - protein, 125 aa, Artificial Sequence
  RVB492 heavy chain variant 2 aa
EVQLVQSGGGLVQPGGSMRLYCAASGFSFSSYAMSWVRQAPGKGLEWVSSLNSIDHRTDYADSVKGRFTISRDNSKNTLYLQMDSLRVEDSAMYYCARGVGLWFGELSWNYFDYWGQGTLVTVSS

SEQ ID NO: 71 - protein, 109 aa, Artificial Sequence
  RVB492 light chain aa
QSALTQPRSVSGSPGQSVTISCTGTSNDIGGYNYVSWYQQHPGKAPKLMIFYVNKRPSGVPDRFSGSKSGNTASLTISGLQAEDEADYYCCSFAGSYSLFGRGTKLTVL

SEQ ID NO: 72 - DNA, 376 bp, Artificial Sequence
  RVB492 heavy chain variant 1 nuc
gaggtgcagctgatggagtctgggggaggcctggtacagccgggggggtccatgagactctactgtgcagcctctggattcagctttagcagctatgccatgagctgggtccgccaggctccagggaaggggctcgagtgggtctcaagtcttaattctattgatcatagaacagactatgcagactccgtgaagggccggttcaccatctccagagacaattccaagaacaccctgtatttacaaatggacagcctgagagtcgaggactcggccatgtattactgtgctcggggggtgggactatggttcggtgaattatcctggaattactttgactactggggccagggaaccctggtcaccgtctcctcag

SEQ ID NO: 73 - DNA, 376 bp, Artificial Sequence
  RVB492 heavy chain variant 2 nuc
gaggtgcagctggtgcagtctgggggaggcctggtacagccgggggggtccatgagactctactgtgcagcctctggattcagctttagcagctatgccatgagctgggtccgccaggctccagggaaggggctcgagtgggtctcaagtcttaattctattgatcatagaacagactatgcagactccgtgaagggccggttcaccatctccagagacaattccaagaacaccctgtatttacaaatggacagcctgagagtcgaggactcggccatgtattactgtgctcggggggtgggactatggttcggtgaattatcctggaattactttgactactggggccagggaaccctggtcaccgtctcctcag

SEQ ID NO: 74 - DNA, 328 bp, Artificial Sequence
  RVB492 light chain nuc
cagtctgccctgactcagcctcgctcagtgtccgggtctcctggacagtcagtcaccatctcctgcactggaaccagcaatgatattggtggttataactatgtctcctggtaccaacaacacccaggcaaagcccccaaactcatgattttttatgtcaataagcggccctcaggggtccctgatcgcttctctggctccaagtctggcaacacggcctccctgaccatctctgggctccaggctgaggatgaagctgattattactgctgctcatttgcaggcagttactccttattcggcagagggaccaagctgaccgtcctag

SEQ ID NO: 75 - protein, 8 aa, Artificial Sequence
  RVC3 CDRH1 aa
TFTFRNYA

SEQ ID NO: 76 - protein, 8 aa, Artificial Sequence
  RVC3 CDRH2 aa
ISASGSST

SEQ ID NO: 77 - protein, 16 aa, Artificial Sequence
  RVC3 CDRH3 aa
AKFAHDFWSGYSYFDS

SEQ ID NO: 78 - protein, 6 aa, Artificial Sequence
  RVC3 CDRL1 aa
QSVNSN

SEQ ID NO: 79 - skipped

SEQ ID NO: 80 - protein, 9 aa, Artificial Sequence
  RVC3 CDRL2 long aa
LIYGASTRA

SEQ ID NO: 81 - protein, 10 aa, Artificial Sequence
  RVC3 CDRL3 aa
QQYNNWVSIT

SEQ ID NO: 82 - DNA, 24 bp, Artificial Sequence
  RVC3 CDRH1 nuc
acattcacgtttagaaactatgcc

SEQ ID NO: 83 - DNA, 24 bp, Artificial Sequence
  RVC3 CDRH2 nuc
attagtgctagtggtagtagcacg

SEQ ID NO: 84 - DNA, 48 bp, Artificial Sequence
  RVC3 CDRH3 nuc
gcgaaatttgctcacgatttttggagtggttattcttactttgactcc

SEQ ID NO: 85 - DNA, 18 bp, Artificial Sequence
  RVC3 CDRL1 nuc
cagagtgttaacagcaac

SEQ ID NO: 86 - skipped

SEQ ID NO: 87 - DNA, 27 bp, Artificial Sequence
  RVC3 CDRL2 long nuc
ctcatctatggtgcatccaccagggcc

SEQ ID NO: 88 - DNA, 30 bp, Artificial Sequence
  RVC3 CDRL3 nuc
cagcagtataataattgggtttcgatcacc

SEQ ID NO: 89 - protein, 123 aa, Artificial Sequence
  RVC3 heavy chain aa
EVQLLESGGGLVQPGGSLRLSCAASTFTFRNYAMSWVRQAPGKGLDWVSGISASGSSTNYAASLKGRFTISRDNSKNTLYLQMNSLRAEDTAVYYCAKFAHDFWSGYSYFDSWGQGTLVTVSS

SEQ ID NO: 90 - protein, 108 aa, Artificial Sequence
  RVC3 light chain aa
EIVMTQSPATLSVSPGERATLSCRAGQSVNSNLAWYQQKPGQAPRLLIYGASTRATGIPARFSGSGSGTEFTLTISSLQSEDFAVYYCQQYNNWVSITFGQGTRLEIK

SEQ ID NO: 91 - DNA, 370 bp, Artificial Sequence
  RVC3 heavy chain nuc
gaggtgcagctgttggagtctgggggaggcctggtgcagccgggggggtccctgagactctcctgtgcagcctctacattcacgtttagaaactatgccatgtcctgggtccgccaggctccagggaaggggctggactgggtctcagggattagtgctagtggtagtagcacgaattatgcagcctccctgaagggccgatttaccatctccagagacaattccaagaacacattgtatctgcaaatgaacagcctgagagccgaggacacggccgtctattactgtgcgaaatttgctcacgatttttggagtggttattcttactttgactcctggggccagggaaccctggtcaccgtctcctcag

SEQ ID NO: 92 - DNA, 325 bp, Artificial Sequence
  RVC3 light chain nuc
gaaatagtgatgacgcagtctccagccaccctgtctgtgtctccaggggaaagagccaccctctcctgcagggccggtcagagtgttaacagcaacttagcctggtaccagcagaaacctgggcaggctcccagactcctcatctatggtgcatccaccagggccactggtatcccagccaggttcagtggcagtgggtctgggacagagttcactctcaccatcagcagcctgcagtctgaagattttgcagtttattactgtcagcagtataataattgggtttcgatcaccttcggccaagggacacgactggagattaaac

SEQ ID NO: 93 - protein, 10 aa, Artificial Sequence
  RVC20 CDRH1 aa
GGSFSSGSYS

SEQ ID NO: 94 - protein, 7 aa, Artificial Sequence
  RVC20 CDRH2 aa
IYYSGST

SEQ ID NO: 95 - protein, 16 aa, Artificial Sequence
  RVC20 CDRH3 aa
ARGTYSDFWSGSPLDY

SEQ ID NO: 96 - protein, 6 aa, Artificial Sequence
  RVC20 CDRL1 aa
QGISNY

SEQ ID NO: 97 - skipped

SEQ ID NO: 98 - protein, 9 aa, Artificial Sequence
  RVC20 CDRL2 long aa
LIYAASSLQ

SEQ ID NO: 99 - protein, 9 aa, Artificial Sequence
  RVC20 CDRL3 aa
QQYDTYPLT

SEQ ID NO: 100 - DNA, 30 bp, Artificial Sequence
  RVC20 CDRH1 nuc
ggtggctccttcagcagtggaagttactcc

SEQ ID NO: 101 - DNA, 21 bp, Artificial Sequence
  RVC20 CDRH2 nuc
atctattacagtgggagcact

SEQ ID NO: 102 - DNA, 48 bp, Artificial Sequence
  RVC20 CDRH3 nuc
gcgagaggcacgtattccgatttttggagtggttcccctttagactac

SEQ ID NO: 103 - DNA, 18 bp, Artificial Sequence
  RVC20 CDRL1 nuc
cagggcattagcaattat

SEQ ID NO: 104 - skipped

SEQ ID NO: 105 - DNA, 27 bp, Artificial Sequence
  RVC20 CDRL2 long nuc
ctgatctatgctgcatccagtttgcaa

SEQ ID NO: 106 - DNA, 27 bp, Artificial Sequence
  RVC20 CDRL3 nuc
caacagtatgatacttaccctctcact

SEQ ID NO: 107 - protein, 124 aa, Artificial Sequence
  RVC20 heavy chain aa
QVQLQESGPGLVKPSQTLSLTCTVSGGSFSSGSYSWNWIRQHPGKGLEWIGYIYYSGSTYYNPSLKSRVTMSVHTSKNQFSLKLNSITAADTAVYYCARGTYSDFWSGSPLDYWGQGTLVTVSS

SEQ ID NO: 108 - protein, 107 aa, Artificial Sequence
  RVC20 light chain aa
DIQMTQSPSSLSASVGDRVTITCRASQGISNYLAWFQQKPGKAPKSLIYAASSLQSGVPSRFSGSGSGTDFTLTINSLQPEDFVTYFCQQYDTYPLTFGGGTKVEIK

SEQ ID NO: 109 - DNA, 373 bp, Artificial Sequence
  RVC20 heavy chain nuc
caggtgcagctgcaggagtcgggcccaggactggtgaagccttcacagaccctgtccctcacctgcactgtctccggtggctccttcagcagtggaagttactcctggaactggatccgccagcacccagggaagggcctggagtggattgggtacatctattacagtgggagcacttattacaacccgtccctcaagagtcgagttaccatgtcagtacacacgtctaagaaccagttctccctgaagctgaactctataactgccgcggacacggccgtgtattactgtgcgagaggcacgtattccgatttttggagtggttcccctttagactactggggccagggaaccctggtcaccgtctcctcag

SEQ ID NO: 110 - DNA, 322 bp, Artificial Sequence
  RVC20 light chain nuc
gacatccagatgacccagtctccatcctcactgtctgcatctgtaggagacagagtcaccatcacttgtcgggcgagtcagggcattagcaattatttagcctggtttcagcagaaaccagggaaagcccctaagtccctgatctatgctgcatccagtttgcaaagtggggtcccatcaaggttcagcggcagtggatctgggacagatttcactctcaccatcaacagcctgcagcctgaagattttgtaacttatttctgccaacagtatgatacttaccctctcactttcggcggagggaccaaggtggagatcaaac

SEQ ID NO: 111 - protein, 10 aa, Artificial Sequence
  RVC21 CDRH1 aa
GGSISNPNYY

SEQ ID NO: 112 - protein, 7 aa, Artificial Sequence
  RVC21 CDRH2 aa
IYYNGYT

SEQ ID NO: 113 - protein, 13 aa, Artificial Sequence
  RVC21 CDRH3 aa
ATQSTMTTIAGHY

SEQ ID NO: 114 - protein, 8 aa, Artificial Sequence
  RVC21 CDRL1 aa
TSNIGNSY

SEQ ID NO: 115 - skipped

SEQ ID NO: 116 - protein, 9 aa, Artificial Sequence
  RVC21 CDRL2 long aa
LIYDNNKRP

SEQ ID NO: 117 - protein, 11 aa, Artificial Sequence
  RVC21 CDRL3 aa
GTWDSSLNAYV

SEQ ID NO: 118 - DNA, 30 bp, Artificial Sequence
  RVC21 CDRH1 nuc
ggtggctccatcagcaaccctaactactac

SEQ ID NO: 119 - DNA, 21 bp, Artificial Sequence
  RVC21 CDRH2 nuc
atctattataatgggtacacc

SEQ ID NO: 120 - DNA, 39 bp, Artificial Sequence
  RVC21 CDRH3 nuc
gcgacgcaatctacgatgactaccatagcgggccactac

SEQ ID NO: 121 - DNA, 24 bp, Artificial Sequence
  RVC21 CDRL1 nuc
acatccaacattgggaattcttat

SEQ ID NO: 122 - skipped

SEQ ID NO: 123 - DNA, 27 bp, Artificial Sequence
  RVC21 CDRL2 long nuc
ctcatttatgacaataataagcgaccc

SEQ ID NO: 124 - DNA, 33 bp, Artificial Sequence
  RVC21 CDRL3 nuc
ggaacatgggacagcagcctgaatgcttatgtc

SEQ ID NO: 125 - protein, 121 aa, Artificial Sequence
  RVC21 heavy chain aa
QLQLQESGPGLVKPSETLSLTCTVSGGSISNPNYYWGWIRQPPGKGLEWIGSIYYNGYTYYNPSLKSRVTISVDKSKDQFFLKMTSLTAADTAVYYCATQSTMTTIAGHYWGQGTLVTVSS

SEQ ID NO: 126 - protein, 110 aa, Artificial Sequence
  RVC21 light chain aa
QSVLTQAPSVSAAPGLKVTISCSGSTSNIGNSYVSWYQQLPGTAPKLLIYDNNKRPSGIPDRFSGSKSDTSATLGITGLQTGDEADYYCGTWDSSLNAYVFGTGTKVTVL

SEQ ID NO: 127 - DNA, 364 bp, Artificial Sequence
  RVC21 heavy chain nuc
cagctgcagctgcaggagtcgggcccaggactggtgaagccttcggagaccctgtccctcacgtgcactgtctctggtggctccatcagcaaccctaactactactggggctggatccgccagcccccagggaagggtctggaatggattgggagtatctattataatgggtacacctactacaacccgtccctcaagagtcgagttaccatatccgtggacaagtccaaggaccagttctttctgaagatgacctctctgaccgccgcagacacggctgtgtattactgtgcgacgcaatctacgatgactaccatagcgggccactactggggccagggaaccctggtcaccgtctcctcag

SEQ ID NO: 128 - DNA, 331 bp, Artificial Sequence
  RVC21 light chain nuc
cagtctgtattgacgcaggcgccctcagtgtctgcggccccaggactaaaggtcaccatctcctgctctggaagcacatccaacattgggaattcttatgtatcctggtaccagcagctcccaggaacagcccccaaactcctcatttatgacaataataagcgaccctcagggattcctgaccgattctctggctccaagtctgacacgtcagccaccctgggcatcaccggactccagactggggacgaggccgattattactgcggaacatgggacagcagcctgaatgcttatgtcttcggaactgggaccaaggtcaccgtcctag

SEQ ID NO: 129 - protein, 8 aa, Artificial Sequence
  RVC38 CDRH1 aa
GGTFSSYA

SEQ ID NO: 130 - protein, 8 aa, Artificial Sequence
  RVC38 CDRH2 aa
IMPMFVAA

SEQ ID NO: 131 - protein, 14 aa, Artificial Sequence
  RVC38 CDRH3 aa
ARGDGYNYKWYFDL

SEQ ID NO: 132 - protein, 6 aa, Artificial Sequence
  RVC38 CDRL1 aa
QDISNY

SEQ ID NO: 133 - skipped

SEQ ID NO: 134 - protein, 9 aa, Artificial Sequence
  RVC38 CDRL2 long aa
LIYAASTLQ

SEQ ID NO: 135 - protein, 10 aa, Artificial Sequence
  RVC38 CDRL3 aa
QQLDTYVALT

SEQ ID NO: 136 - DNA, 24 bp, Artificial Sequence
  RVC38 CDRH1 nuc
ggaggcaccttcagcagctatgcc

SEQ ID NO: 137 - DNA, 24 bp, Artificial Sequence
  RVC38 CDRH2 nuc
atcatgcctatgtttgtggcggca

SEQ ID NO: 138 - DNA, 42 bp, Artificial Sequence
  RVC38 CDRH3 nuc
gcgagaggggatggctacaattacaagtggtattttgacctt

SEQ ID NO: 139 - DNA, 18 bp, Artificial Sequence
  RVC38 CDRL1 nuc
caggacattagtaattat

SEQ ID NO: 140 - skipped

SEQ ID NO: 141 - DNA, 27 bp, Artificial Sequence
  RVC38 CDRL2 long nuc
ctgatctatgctgcatccactttgcaa

SEQ ID NO: 142 - DNA, 30 bp, Artificial Sequence
  RVC38 CDRL3 nuc
caacagcttgatacttacgtcgcgctcact

SEQ ID NO: 143 - protein, 121 aa, Artificial Sequence
  RVC38 heavy chain aa
EVQLVQSGAEVKKPGSSVRVSCKASGGTFSSYAISWVRQAPGLGLEWMGGIMPMFVAANYAQNFQGRVTVSVDKSTNTAYMEMHNLRSDDTAMYYCARGDGYNYKWYFDLWGQGTLVTVSS

SEQ ID NO: 144 - protein, 108 aa, Artificial Sequence
  RVC38 light chain aa
DIQLTQSPSFLSASVGDRVTITCRASQDISNYLAWYQQKPGKPPKLLIYAASTLQRGVPSRFSGSGSGSEFTLTISSLQPEDFATYYCQQLDTYVALTFGGGTKVEIK

SEQ ID NO: 145 - DNA, 364 bp, Artificial Sequence
  RVC38 heavy chain nuc
gaggtgcagctggtgcagtctggggctgaggtgaagaagcctgggtcctcggtgagggtctcctgcaaggcttctggaggcaccttcagcagctatgccatcagctgggtgcgacaggcccctgggctagggcttgagtggatgggagggatcatgcctatgtttgtggcggcaaactacgcacagaacttccagggcagagtcacggtttctgtggacaaatccacgaacaccgcctatatggagatgcacaacctgagatctgacgacacggccatgtattactgtgcgagaggggatggctacaattacaagtggtattttgacctttggggccagggaaccctagtcaccgtctcctcag

SEQ ID NO: 146 - DNA, 325 bp, Artificial Sequence
  RVC38 light chain nuc
gacatccagttgacccagtctccatccttcctgtctgcatctgtaggagacagagtcaccatcacttgccgggccagtcaggacattagtaattatttagcctggtatcagcaaaaaccagggaagccccctaaactcctgatctatgctgcatccactttgcaaaggggggtcccatcaaggttcagtggcagtggatctgggtcagaattcactctcacaatcagcagcctgcagcctgaagattttgcaacttattactgtcaacagcttgatacttacgtcgcgctcactttcggcggagggaccaaggtggagatcaaac

SEQ ID NO: 147 - protein, 8 aa, Artificial Sequence
  RVC44 CDRH1 aa
GFTFSSYS

SEQ ID NO: 148 - protein, 8 aa, Artificial Sequence
  RVC44 CDRH2 aa
ISTTGTYI

SEQ ID NO: 149 - protein, 17 aa, Artificial Sequence
  RVC44 CDRH3 aa
ARRSAIALAGTQRAFDI

SEQ ID NO: 150 - protein, 6 aa, Artificial Sequence
  RVC44 CDRL1 aa
QNINNY

SEQ ID NO: 151 - skipped

SEQ ID NO: 152 - protein, 9 aa, Artificial Sequence
  RVC44 CDRL2 long aa
LIYAASSLH

SEQ ID NO: 153 - protein, 9 aa, Artificial Sequence
  RVC44 CDRL3 aa
QQSYSNPWT

SEQ ID NO: 154 - DNA, 24 bp, Artificial Sequence
  RVC44 CDRH1 nuc
ggcttcacctttagtagttatagt

SEQ ID NO: 155 - DNA, 24 bp, Artificial Sequence
  RVC44 CDRH2 nuc
atcagtactactggtacttacata

SEQ ID NO: 156 - DNA, 51 bp, Artificial Sequence
  RVC44 CDRH3 nuc
gcgagacggtcggccatagcactggctggtacgcagcgtgcttttgatatc

SEQ ID NO: 157 - DNA, 18 bp, Artificial Sequence
  RVC44 CDRL1 nuc
cagaacattaacaactat

SEQ ID NO: 158 - skipped

SEQ ID NO: 159 - DNA, 27 bp, Artificial Sequence
  RVC44 CDRL2 long nuc
ctgatctatgctgcatccagtttacat

SEQ ID NO: 160 - DNA, 27 bp, Artificial Sequence
  RVC44 CDRL3 nuc
caacagagttacagtaacccttggacg

SEQ ID NO: 161 - protein, 124 aa, Artificial Sequence
  RVC44 heavy chain aa
EVQLVQSGGGLVKPGGSLRLSCAASGFTFSSYSMSWVRQAPGKGLEWVSSISTTGTYIYYADSVEGRFSISRDSARSSLFLQMNSLRAEDTAVYYCARRSAIALAGTQRAFDIWGPGTNVIVSS

SEQ ID NO: 162 - protein, 107 aa, Artificial Sequence
  RVC44 light chain aa
DIQMTQSPSSLSASVGDRVTITCRASQNINNYLNWYQQKLGKAPKLLIYAASSLHSGVPSRFSASGSGTDFILTISNLQPEDCATYYCQQSYSNPWTFGQGTKVEIK

SEQ ID NO: 163 - DNA, 373 bp, Artificial Sequence
  RVC44 heavy chain nuc
gaggtgcagctggtgcagtctgggggaggcctggtcaagcctggggggtccctgagactctcctgtgcagcctctggcttcacctttagtagttatagtatgagttgggtccgccaggctccagggaagggcctggagtgggtctcatccatcagtactactggtacttacatatactacgcagactcagtggagggccgattctccatttccagagacagcgccaggagctctctgtttctgcaaatgaacagcctgagagccgaggacacggctgtctattactgtgcgagacggtcggccatagcactggctggtacgcagcgtgcttttgatatctggggcccagggacaaacgtcatcgtctcttcag

SEQ ID NO: 164 - DNA, 322 bp, Artificial Sequence
  RVC44 light chain nuc
gacatccagatgacccagtctccatcttccctgtctgcatctgtaggagacagagtcaccatcacttgccgggcaagtcagaacattaacaactatttaaattggtatcagcagaaactagggaaagcccctaagctcctgatctatgctgcatccagtttacatagtggggtcccatcaaggttcagtgccagtggatctgggacagatttcattctgaccatcagtaatctgcaacctgaagattgtgcaacttactactgtcaacagagttacagtaacccttggacgttcggccaagggaccaaggtggaaatcaaac

SEQ ID NO: 165 - protein, 8 aa, Artificial Sequence
  RVC58 CDRH1 aa
GFTFSTYA

SEQ ID NO: 166 - protein, 8 aa, Artificial Sequence
  RVC58 CDRH2 aa
ISDRGGSR

SEQ ID NO: 167 - protein, 17 aa, Artificial Sequence
  RVC58 CDRH3 aa
ARDIAPPYNYYFYGMDV

SEQ ID NO: 168 - protein, 9 aa, Artificial Sequence
  RVC58 CDRL1 aa
SSDIGAFNY

SEQ ID NO: 169 - skipped

SEQ ID NO: 170 - protein, 9 aa, Artificial Sequence
  RVC58 CDRL2 long aa
IIYEVSNRP

SEQ ID NO: 171 - protein, 10 aa, Artificial Sequence
  RVC58 CDRL3 aa
NSYTSSSTQL

SEQ ID NO: 172 - DNA, 24 bp, Artificial Sequence
  RVC58 CDRH1 nuc
ggattcacctttagcacctatgcc

SEQ ID NO: 173 - DNA, 24 bp, Artificial Sequence
  RVC58 CDRH2 nuc
attagtgatagaggtggtagtaga

SEQ ID NO: 174 - DNA, 51 bp, Artificial Sequence
  RVC58 CDRH3 nuc
gcgagagatattgcccccccatataactactacttctacggtatggacgtc

SEQ ID NO: 175 - DNA, 27 bp, Artificial Sequence
  RVC58 CDRL1 nuc
agcagtgacattggtgcttttaactat

SEQ ID NO: 176 - skipped

SEQ ID NO: 177 - DNA, 27 bp, Artificial Sequence
  RVC58 CDRL2 long nuc
ataatttatgaggtcagtaatcggccc

SEQ ID NO: 178 - DNA, 30 bp, Artificial Sequence
  RVC58 CDRL3 nuc
aactcatatacaagcagcagcactcagtta

SEQ ID NO: 179 - protein, 124 aa, Artificial Sequence
  RVC58 heavy chain aa
EVQLVESGGGLVQPGGSLRLSCAASGFTFSTYAMNWVRQAPGKGLEWVSGISDRGGSRYYAGSVKGRFTISRDNSKNTLFLQMNSLRAEDTAVYYCARDIAPPYNYYFYGMDVWGRGTTVTVSS

SEQ ID NO: 180 - protein, 110 aa, Artificial Sequence
  RVC58 light chain aa
QSALTQPASVSGSPGQSITISCTGTSSDIGAFNYVSWYQQHPGKAPKLIIYEVSNRPSGVSNRFSGSKSGNTASLTISGLQAEDEADYYCNSYTSSSTQLFGGGTKLTVL

SEQ ID NO: 181 - DNA, 373 bp, Artificial Sequence
  RVC58 heavy chain nuc
gaggtgcagctggtggagtctgggggaggcttggtacagcctggggggtccctgagactctcctgtgcggcctctggattcacctttagcacctatgccatgaattgggtccgccaggctccagggaaggggctggagtgggtctcaggtattagtgatagaggtggtagtagatactacgcaggctccgtgaagggccggttcaccatctccagagacaattccaagaacacgctgtttctgcaaatgaacagcctgagagccgaggacacggccgtatattactgtgcgagagatattgcccccccatataactactacttctacggtatggacgtctggggccgagggaccacggtcaccgtctcctcag

SEQ ID NO: 182 - DNA, 331 bp, Artificial Sequence
  RVC58 light chain nuc
cagtctgccctgactcagcctgcctccgtgtctgggtctcctggacagtcgatcaccatctcctgcactggtaccagcagtgacattggtgcttttaactatgtctcttggtaccaacagcacccaggcaaagcccccaaactcataatttatgaggtcagtaatcggccctcaggggtttctaatcgcttctctggctccaagtctggcaacacggcctccctgaccatctctgggctccaggctgaggacgaggctgattattactgcaactcatatacaagcagcagcactcagttattcggcggagggaccaagctgaccgtcctag

SEQ ID NO: 183 - protein, 8 aa, Artificial Sequence
  RVC68 CDRH1 aa
GGSISEHH

SEQ ID NO: 184 - protein, 7 aa, Artificial Sequence
  RVC68 CDRH2 aa
IFHSGST

SEQ ID NO: 185 - protein, 14 aa, Artificial Sequence
  RVC68 CDRH3 aa
ARAVSTYYYYYIDV

SEQ ID NO: 186 - protein, 6 aa, Artificial Sequence
  RVC68 CDRL1 aa
QDISNW

SEQ ID NO: 187 - skipped

SEQ ID NO: 188 - protein, 9 aa, Artificial Sequence
  RVC68 CDRL2 long aa
LIYAASSLQ

SEQ ID NO: 189 - protein, 9 aa, Artificial Sequence
  RVC68 CDRL3 aa
QQAKSFPLT

SEQ ID NO: 190 - DNA, 24 bp, Artificial Sequence
  RVC68 CDRH1 nuc
ggtggctccattagtgagcaccac

SEQ ID NO: 191 - DNA, 21 bp, Artificial Sequence
  RVC68 CDRH2 nuc
atctttcacagtgggagtacc

SEQ ID NO: 192 - DNA, 42 bp, Artificial Sequence
  RVC68 CDRH3 nuc
gcgagagcggtgtctacttactactactattacatagacgtc

SEQ ID NO: 193 - DNA, 18 bp, Artificial Sequence
  RVC68 CDRL1 nuc
caggatattagcaactgg

SEQ ID NO: 194 - skipped

SEQ ID NO: 195 - DNA, 27 bp, Artificial Sequence
  RVC68 CDRL2 long nuc
ctgatctatgctgcgtccagtttgcaa

SEQ ID NO: 196 - DNA, 27 bp, Artificial Sequence
  RVC68 CDRL3 nuc
caacaggctaagagtttccctcttact

SEQ ID NO: 197 - protein, 120 aa, Artificial Sequence
  RVC68 heavy chain aa
QVQLQESGPRLVKPSETLSLTCTFSGGSISEHHWSWLRQSPGKGLEWIGYIFHSGSTNYNPSLKSRVNISLDKSKNQFSLKLSSVTAADTAVYFCARAVSTYYYYYIDVWGQGTTVTVSS

SEQ ID NO: 198 - protein, 107 aa, Artificial Sequence
  RVC68 light chain aa
DIQMTQSPSSVSASVGDRVTITCRASQDISNWLAWYQQKPGKAPKLLIYAASSLQSGISSRFSGGGSGTDFTLTISSLQPEDFASYYCQQAKSFPLTFGQGTKLEIK

SEQ ID NO: 199 - DNA, 361 bp, Artificial Sequence
  RVC68 heavy chain nuc
caggtgcagctacaggagtcgggcccaagactggtgaagccctcggagaccctgtccctcacctgcactttctctggtggctccattagtgagcaccactggagctggctccggcagtccccagggaagggactggagtggattggatatatctttcacagtgggagtaccaactacaacccctccctcaagagtcgagtcaacatatcattagacaagtccaagaaccagttctccctgaagctgagttctgtgaccgctgcggacacggccgtgtatttctgtgcgagagcggtgtctacttactactactattacatagacgtctggggccaagggaccacggtcaccgtctcctcag

SEQ ID NO: 200 - DNA, 322 bp, Artificial Sequence
  RVC68 light chain nuc
gacatccagatgacccagtctccatcttccgtgtctgcatctgtaggagacagagtcaccatcacttgtcgggcgagtcaggatattagcaactggttagcctggtatcagcagaaaccagggaaagcccctaaactcctgatctatgctgcgtccagtttgcaaagtgggatctcatctaggttcagcggcggtggctctgggacagatttcactctcaccatcagcagcctgcagcctgaagattttgcaagttactactgtcaacaggctaagagtttccctcttacttttggccaggggaccaagctggagatcaaac

SEQ ID NO: 201 - protein, 8 aa, Artificial Sequence
  RVC111 CDRH1 aa
GFSFSSYV

SEQ ID NO: 202 - protein, 8 aa, Artificial Sequence
  RVC111 CDRH2 aa
ISYDGSNK

SEQ ID NO: 203 - protein, 13 aa, Artificial Sequence
  RVC111 CDRH3 aa
ARGSGTQTPLFDY

SEQ ID NO: 204 - protein, 6 aa, Artificial Sequence
  RVC111 CDRL1 aa
QSITSW

SEQ ID NO: 205 - skipped

SEQ ID NO: 206 - protein, 9 aa, Artificial Sequence
  RVC111 CDRL2 long aa
LIYDDSTLE

SEQ ID NO: 207 - protein, 9 aa, Artificial Sequence
  RVC111 CDRL3 aa
QQYESYSGT

SEQ ID NO: 208 - DNA, 24 bp, Artificial Sequence
  RVC111 CDRH1 nuc
ggattctccttcagtagctatgtt

SEQ ID NO: 209 - DNA, 24 bp, Artificial Sequence
  RVC111 CDRH2 nuc
atatcatatgatggaagtaataaa

SEQ ID NO: 210 - DNA, 39 bp, Artificial Sequence
  RVC111 CDRH3 nuc
gcgagagggtccggaacccaaactcccctctttgactac

SEQ ID NO: 211 - DNA, 18 bp, Artificial Sequence
  RVC111 CDRL1 nuc
cagagtattactagctgg

SEQ ID NO: 212 - skipped

SEQ ID NO: 213 - DNA, 27 bp, Artificial Sequence
  RVC111 CDRL2 long nuc
ctgatctatgatgactccactttggaa

SEQ ID NO: 214 - DNA, 27 bp, Artificial Sequence
  RVC111 CDRL3 nuc
caacagtatgagagttattcagggacg

SEQ ID NO: 215 - protein, 120 aa, Artificial Sequence
  RVC111 heavy chain aa
QVQLVESGGGVVQPGRSLRLSCAASGFSFSSYVMYWVRQAPGKGLEWVTIISYDGSNKYYADSVKGRFTISRDNSKNTLYLQMNSLRAEDTAVYYCARGSGTQTPLFDYWGQGTLVTVSS

SEQ ID NO: 216 - protein, 107 aa, Artificial Sequence
  RVC111 light chain aa
DIQMTQSPSTLSASVGDRVTITCRANQSITSWVAWYQQMPGRAPKLLIYDDSTLESGVPSRFSGSGSGTEFTLTISSLQPDDFATYYCQQYESYSGTFGQGTKVEIK

SEQ ID NO: 217 - DNA, 361 bp, Artificial Sequence
  RVC111 heavy chain nuc
caggtgcaactggtggagtctgggggaggcgtggtccagcctgggaggtccctgagactctcctgtgcagcctctggattctccttcagtagctatgttatgtactgggtccgccaggctccaggcaaggggctggagtgggtgacaattatatcatatgatggaagtaataaatactacgcagactccgtgaagggccgattcaccatctccagagacaattccaagaacacgctgtatctgcaaatgaacagcctgagagctgaggacacggctgtctattactgtgcgagagggtccggaacccaaactcccctctttgactactggggccagggaaccctggtcaccgtctcctcag

SEQ ID NO: 218 - DNA, 322 bp, Artificial Sequence
  RVC111 light chain nuc
gacatccagatgacccagtctccttccaccctgtctgcatctgtgggagacagagtcaccatcacttgccgggccaatcagagtattactagctgggtggcctggtatcagcagatgccagggagagcccctaaactcctgatctatgatgactccactttggaaagtggggtcccatcaaggttcagcggcagtggatctgggacagaattcactctcaccatcagcagcctgcagcctgatgattttgcaacttattactgccaacagtatgagagttattcagggacgttcggccaagggaccaaggtggaaatcaaac